European Patent Application EP 4 649 965 A1, published November 19, 2025. Title: COMPOSITION FOR THE TARGETED IMAGING OF CARCINOMA. Applicant: ONCOPOLE CLAUDIUS REGAUD. The sequence listing filed with the application follows.

SEQUENCE LISTING (2 sequences)

SEQ ID NO: 1 - protein, 143 aa, synthetic construct
MSYSITLRVYQTNRDRGYFSIVEKTVWHFANGGTWSECNGAHTLTQGGSGTSGVLRFLSTKGERITVAVGVHNYKRWCDVVTGLKPDETALVINPQYYNNGGRDYVREKQLAEYSVTSAIGTKVEVVYTVAEGNNLEANVIFS

SEQ ID NO: 2 - DNA, 432 bp, synthetic construct
  source 1..432: mol_type = other DNA
atgtcttacagtattaccctccgtgtctaccagaccaaccgcgatcgcgggtacttctccatcgttgagaagaccgtttggcactttgccaacggtggtacttggtccgagtgcaacggcgcccacaccctcacccagggtggtagcggcacgtctggagttcttcgtttcttgtcgaccaagggcgagcgcatcactgtcgctgtcggggtgcacaactacaagcgttggtgcgacgtcgtcactgggcttaagcccgacgagaccgctctggtgatcaacccgcagtactacaacaacggaggacgggactatgtcagggagaaacaattggctgagtacagcgtcacgagcgccattggaacgaaagtcgaagttgtttacaccgtcgctgaaggcaacaatctcgaggccaacgtcatcttctcttga